European Patent Specification EP 3 848 054 B1, published January 29, 2025. Title: Novel Cyclic Dinucleotide Derivatives and Antibody-Drug Conjugate thereof. Applicant: DAIICHI SANKYO COMPANY, LIMITED. The sequence listing filed with the application follows.

SEQUENCE LISTING (36 sequences)

SEQ ID NO: 1 - protein, 214 aa, Artificial Sequence
  Trastuzumab Light Chain
DIQMTQSPSSLSASVGDRVTITCRASQDVNTAVAWYQQKPGKAPKLLIYSASFLYSGVPSRFSGSRSGTDFTLTISSLQPEDFATYYCQQHYTTPPTFGQGTKVEIKRTVAAPSVFIFPPSDEQLKSGTASVVCLLNNFYPREAKVQWKVDNALQSGNSQESVTEQDSKDSTYSLSSTLTLSKADYEKHKVYACEVTHQGLSSPVTKSFNRGEC

SEQ ID NO: 2 - protein, 450 aa, Artificial Sequence
  Trastuzumab Heavy Chain
EVQLVESGGGLVQPGGSLRLSCAASGFNIKDTYIHWVRQAPGKGLEWVARIYPTNGYTRYADSVKGRFTISADTSKNTAYLQMNSLRAEDTAVYYCSRWGGDGFYAMDYWGQGTLVTVSSASTKGPSVFPLAPSSKSTSGGTAALGCLVKDYFPEPVTVSWNSGALTSGVHTFPAVLQSSGLYSLSSVVTVPSSSLGTQTYICNVNHKPSNTKVDKKVEPKSCDKTHTCPPCPAPELLGGPSVFLFPPKPKDTLMISRTPEVTCVVVDVSHEDPEVKFNWYVDGVEVHNAKTKPREEQYNSTYRVVSVLTVLHQDWLNGKEYKCKVSNKALPAPIEKTISKAKGQPREPQVYTLPPSREEMTKNQVSLTCLVKGFYPSDIAVEWESNGQPENNYKTTPPVLDSDGSFFLYSKLTVDKSRWQQGNVFSCSVMHEALHNHYTQKSLSLSPGK

SEQ ID NO: 3 - protein, 450 aa, Artificial Sequence
  Modified HER2 antibody Heavy Chain
EVQLVESGGGLVQPGGSLRLSCAASGFNIKDTYIHWVRQAPGKGLEWVARIYPTNGYTRYADSVKGRFTISADTSKNTAYLQMNSLRAEDTAVYYCSRWGGDGFYAMDYWGQGTLVTVSSASTKGPSVFPLAPSSKSTSGGTAALGCLVKDYFPEPVTVSWNSGALTSGVHTFPAVLQSSGLYSLSSVVTVPSSSLGTQTYICNVNHKPSNTKVDKKVEPKSCDKTHTCPPCPAPEAAGGPSVFLFPPKPKDTLMISRTPEVTCVVVDVSHEDPEVKFNWYVDGVEVHNAKTKPREEQYNSTYRVVSVLTVLHQDWLNGKEYKCKVSNKALPAPIEKTISKAKGQPREPQVYTLPPSREEMTKNQVSLTCLVKGFYPSDIAVEWESNGQPENNYKTTPPVLDSDGSFFLYSKLTVDKSRWQQGNVFSCSVMHEALHNHYTQKSLSLSPGK

SEQ ID NO: 4 - protein, 379 aa, Homo sapiens [sequence omitted]

SEQ ID NO: 5 - DNA, 1140 bp, Homo sapiens
atgccccactccagcctgcatccatccatcccgtgtcccaggggtcacggggcccagaaggcagccttggttctgctgagtgcctgcctggtgaccctttgggggctaggagagccaccagagcacactctccggtacctggtgctccacctagcctccctgcagctgggactgctgttaaacggggtctgcagcctggctgaggagctgcgccacatccactccaggtaccggggcagctactggaggactgtgcgggcctgcctgggctgccccctccgccgtggggccctgttgctgctgtccatctatttctactactccctcccaaatgcggtcggcccgcccttcacttggatgcttgccctcctgggcctctcgcaggcactgaacatcctcctgggcctcaagggcctggccccagctgagatctctgcagtgtgtgaaaaagggaatttcaacgtggcccatgggctggcatggtcatattacatcggatatctgcggctgatcctgccagagctccaggcccggattcgaacttacaatcagcattacaacaacctgctacggggtgcagtgagccagcggctgtatattctcctcccattggactgtggggtgcctgataacctgagtatggctgaccccaacattcgcttcctggataaactgccccagcagaccggtgaccatgctggcatcaaggatcgggtttacagcaacagcatctatgagcttctggagaacgggcagcgggcgggcacctgtgtcctggagtacgccacccccttgcagactttgtttgccatgtcacaatacagtcaagctggctttagccgggaggataggcttgagcaggccaaactcttctgccggacacttgaggacatcctggcagatgcccctgagtctcagaacaactgccgcctcattgcctaccaggaacctgcagatgacagcagcttctcgctgtcccaggaggttctccggcacctgcggcaggaggaaaaggaagaggttactgtgggcagcttgaagacctcagcggtgcccagtacctccacgatgtcccaagagcctgagctcctcatcagtggaatggaaaagcccctccctctccgcacggatttctcttag

SEQ ID NO: 6 - protein, 379 aa, Homo sapiens
MPHSSLHPSIPCPRGHGAQKAALVLLSACLVTLWGLGEPPEHTLRYLVLHLASLQLGLLLNGVCSLAEELRHIHSRYRGSYWRTVRACLGCPLRRGALLLLSIYFYYSLPNAVGPPFTWMLALLGLSQALNILLGLKGLAPAEISAVCEKGNFNVAHGLAWSYYIGYLRLILPELQARIRTYNQHYNNLLRGAVSQRLYILLPLDCGVPDNLSMADPNIRFLDKLPQQTGDHAGIKDRVYSNSIYELLENGQRAGTCVLEYATPLQTLFAMSQYSQAGFSREDRLEQAKLFCRTLEDILADAPESQNNCRLIAYQEPADDSSFSLSQEVLRHLRQEEKEEVTVGSLKTSAVPSTSTMSQEPELLISGMEKPLPLRTDFS

SEQ ID NO: 7 - DNA, 1140 bp, Homo sapiens
atgccccactccagcctgcatccatccatcccgtgtcccaggggtcacggggcccagaaggcagccttggttctgctgagtgcctgcctggtgaccctttgggggctaggagagccaccagagcacactctccggtacctggtgctccacctagcctccctgcagctgggactgctgttaaacggggtctgcagcctggctgaggagctgcgccacatccactccaggtaccggggcagctactggaggactgtgcgggcctgcctgggctgccccctccgccgtggggccctgttgctgctgtccatctatttctactactccctcccaaatgcggtcggcccgcccttcacttggatgcttgccctcctgggcctctcgcaggcactgaacatcctcctgggcctcaagggcctggccccagctgagatctctgcagtgtgtgaaaaagggaatttcaacgtggcccatgggctggcatggtcatattacatcggatatctgcggctgatcctgccagagctccaggcccggattcgaacttacaatcagcattacaacaacctgctacggggtgcagtgagccagcggctgtatattctcctcccattggactgtggggtgcctgataacctgagtatggctgaccccaacattcgcttcctggataaactgccccagcagaccggtgaccgtgctggcatcaaggatcgggtttacagcaacagcatctatgagcttctggagaacgggcagcgggcgggcacctgtgtcctggagtacgccacccccttgcagactttgtttgccatgtcacaatacagtcaagctggctttagccgggaggataggcttgagcaggccaaactcttctgccggacacttgaggacatcctggcagatgcccctgagtctcagaacaactgccgcctcattgcctaccaggaacctgcagatgacagcagcttctcgctgtcccaggaggttctccggcacctgcggcaggaggaaaaggaagaggttactgtgggcagcttgaagacctcagcggtgcccagtacctccacgatgtcccaagagcctgagctcctcatcagtggaatggaaaagcccctccctctccgcacggatttctcttag

SEQ ID NO: 8 - protein, 379 aa, Homo sapiens
MPHSSLHPSIPCPRGHGAQKAALVLLSACLVTLWGLGEPPEHTLRYLVLHLASLQLGLLLNGVCSLAEELHHIHSRYRGSYWRTVRACLGCPLRRGALLLLSIYFYYSLPNAVGPPFTWMLALLGLSQALNILLGLKGLAPAEISAVCEKGNFNVAHGLAWSYYIGYLRLILPELQARIRTYNQHYNNLLRGAVSQRLYILLPLDCGVPDNLSMADPNIRFLDKLPQQTADRAGIKDRVYSNSIYELLENGQRAGTCVLEYATPLQTLFAMSQYSQAGFSREDRLEQAKLFCQTLEDILADAPESQNNCRLIAYQEPADDSSFSLSQEVLRHLRQEEKEEVTVGSLKTSAVPSTSTMSQEPELLISGMEKPLPLRTDFS

SEQ ID NO: 9 - DNA, 1140 bp, Homo sapiens
atgccccactccagcctgcatccatccatcccgtgtcccaggggtcacggggcccagaaggcagccttggttctgctgagtgcctgcctggtgaccctttgggggctaggagagccaccagagcacactctccggtacctggtgctccacctagcctccctgcagctgggactgctgttaaacggggtctgcagcctggctgaggagctgcaccacatccactccaggtaccggggcagctactggaggactgtgcgggcctgcctgggctgccccctccgccgtggggccctgttgctgctgtccatctatttctactactccctcccaaatgcggtcggcccgcccttcacttggatgcttgccctcctgggcctctcgcaggcactgaacatcctcctgggcctcaagggcctggccccagctgagatctctgcagtgtgtgaaaaagggaatttcaacgtggcccatgggctggcatggtcatattacatcggatatctgcggctgatcctgccagagctccaggcccggattcgaacttacaatcagcattacaacaacctgctacggggtgcagtgagccagcggctgtatattctcctcccattggactgtggggtgcctgataacctgagtatggctgaccccaacattcgcttcctggataaactgccccagcagaccgctgaccgtgctggcatcaaggatcgggtttacagcaacagcatctatgagcttctggagaacgggcagcgggcgggcacctgtgtcctggagtacgccacccccttgcagactttgtttgccatgtcacaatacagtcaagctggctttagccgggaggataggcttgagcaggccaaactcttctgccagacacttgaggacatcctggcagatgcccctgagtctcagaacaactgccgcctcattgcctaccaggaacctgcagatgacagcagcttctcgctgtcccaggaggttctccggcacctgcggcaggaggaaaaggaagaggttactgtgggcagcttgaagacctcagcggtgcccagtacctccacgatgtcccaagagcctgagctcctcatcagtggaatggaaaagcccctccctctccgcacggatttctcttag

SEQ ID NO: 10 - protein, 378 aa, Mus musculus
MPYSNLHPAIPRPRGHRSKYVALIFLVASLMILWVAKDPPNHTLKYLALHLASHELGLLLKNLCCLAEELCHVQSRYQGSYWKAVRACLGCPIHCMAMILLSSYFYFLQNTADIYLSWMFGLLVLYKSLSMLLGLQSLTPAEVSAVCEEKKLNVAHGLAWSYYIGYLRLILPGLQARIRMFNQLHNNMLSGAGSRRLYILFPLDCGVPDNLSVVDPNIRFRDMLPQQNIDRAGIKNRVYSNSVYEILENGQPAGVCILEYATPLQTLFAMSQDAKAGFSREDRLEQAKLFCRTLEEILEDVPESRNNCRLIVYQEPTDGNSFSLSQEVLRHIRQEEKEEVTMNAPMTSVAPPPSVLSQEPRLLISGMDQPLPLRTDLI

SEQ ID NO: 11 - DNA, 1137 bp, Mus musculus
atgccatactccaacctgcatccagccatcccacggcccagaggtcaccgctccaaatatgtagccctcatctttctggtggccagcctgatgatcctttgggtggcaaaggatccaccaaatcacactctgaagtacctagcacttcacctagcctcgcacgaacttggactactgttgaaaaacctctgctgtctggctgaagagctgtgccatgtccagtccaggtaccagggcagctactggaaggctgtgcgcgcctgcctgggatgccccatccactgtatggctatgattctactatcgtcttatttctatttcctccaaaacactgctgacatatacctcagttggatgtttggccttctggtcctctataagtccctaagcatgctcctgggccttcagagcttgactccagcggaagtctctgcagtctgtgaagaaaagaagttaaatgttgcccacgggctggcctggtcatactacattgggtacttgcggttgatcttaccagggctccaggcccggatccgaatgttcaatcagctacataacaacatgctcagtggtgcagggagccgaagactgtacatcctctttccattggactgtggggtgcctgacaacctgagtgtagttgaccccaacattcgattccgagatatgctgccccagcaaaacatcgaccgtgctggcatcaagaatcgggtttattccaacagcgtctacgagattctggagaacggacagccagcaggcgtctgtatcctggagtacgccacccccttgcagaccctgtttgccatgtcacaggatgccaaagctggcttcagtcgggaggatcggcttgagcaggctaaactcttctgccggacacttgaggaaatcctggaagatgtccccgagtctcgaaataactgccgcctcattgtctaccaagaacccacagacggaaacagtttctcactgtctcaggaggtgctccggcacattcgtcaggaagaaaaggaggaggttaccatgaatgcccccatgacctcagtggcacctcctccctccgtactgtcccaagagccaagactcctcatcagtggtatggatcagcctctcccactccgcactgacctcatctga

SEQ ID NO: 12 - DNA, 27 bp, Artificial Sequence
  primer
cgtgctggcatcaaggatcgggtttac

SEQ ID NO: 13 - DNA, 27 bp, Artificial Sequence
  primer
gtcaccggtctgctggggcagtttatc

SEQ ID NO: 14 - DNA, 33 bp, Artificial Sequence
  primer
gctgaccgtgctggcatcaaggatcgggtttac

SEQ ID NO: 15 - DNA, 25 bp, Artificial Sequence
  primer
ggtctgctggggcagtttatccagg

SEQ ID NO: 16 - DNA, 24 bp, Artificial Sequence
  primer
caccacatccactccaggtaccgg

SEQ ID NO: 17 - DNA, 24 bp, Artificial Sequence
  primer
cagctcctcagccaggctgcagac

SEQ ID NO: 18 - DNA, 25 bp, Artificial Sequence
  primer
cagacacttgaggacatcctggcag

SEQ ID NO: 19 - DNA, 23 bp, Artificial Sequence
  primer
gcagaagagtttggcctgctcaa

SEQ ID NO: 20 - DNA, 39 bp, Artificial Sequence
  primer
acctgtattttcagggcctggccccagctgagatctctg

SEQ ID NO: 21 - DNA, 44 bp, Artificial Sequence
  primer
cagaattcgcaagcttttaagtaacctcttccttttcctcctgc

SEQ ID NO: 22 - protein, 243 aa, Artificial Sequence
  HisAviTEV-hSTING (139-342) human WT
MGSSHHHHHHSSGSGLNDIFEAQKIEWHEGGSENLYFQGLAPAEISAVCEKGNFNVAHGLAWSYYIGYLRLILPELQARIRTYNQHYNNLLRGAVSQRLYILLPLDCGVPDNLSMADPNIRFLDKLPQQTGDRAGIKDRVYSNSIYELLENGQRAGTCVLEYATPLQTLFAMSQYSQAGFSREDRLEQAKLFCRTLEDILADAPESQNNCRLIAYQEPADDSSFSLSQEVLRHLRQEEKEEVT

SEQ ID NO: 23 - protein, 243 aa, Artificial Sequence
  HisAviTEV-hSTING (139-342) human REF mutant
MGSSHHHHHHSSGSGLNDIFEAQKIEWHEGGSENLYFQGLAPAEISAVCEKGNFNVAHGLAWSYYIGYLRLILPELQARIRTYNQHYNNLLRGAVSQRLYILLPLDCGVPDNLSMADPNIRFLDKLPQQTGDHAGIKDRVYSNSIYELLENGQRAGTCVLEYATPLQTLFAMSQYSQAGFSREDRLEQAKLFCRTLEDILADAPESQNNCRLIAYQEPADDSSFSLSQEVLRHLRQEEKEEVT

SEQ ID NO: 24 - protein, 243 aa, Artificial Sequence
  HisAviTEV-hSTING (139-342) human AQ mutant
MGSSHHHHHHSSGSGLNDIFEAQKIEWHEGGSENLYFQGLAPAEISAVCEKGNFNVAHGLAWSYYIGYLRLILPELQARIRTYNQHYNNLLRGAVSQRLYILLPLDCGVPDNLSMADPNIRFLDKLPQQTADRAGIKDRVYSNSIYELLENGQRAGTCVLEYATPLQTLFAMSQYSQAGFSREDRLEQAKLFCQTLEDILADAPESQNNCRLIAYQEPADDSSFSLSQEVLRHLRQEEKEEVT

SEQ ID NO: 25 - protein, 243 aa, Artificial Sequence
  HisAviTEV-hSTING (139-342) mouse WT
MGSSHHHHHHSSGSGLNDIFEAQKIEWHEGGSENLYFQGLTPAEVSAVCEEKKLNVAHGLAWSYYIGYLRLILPGLQARIRMFNQLHNNMLSGAGSRRLYILFPLDCGVPDNLSVVDPNIRFRDMLPQQNIDRAGIKNRVYSNSVYEILENGQPAGVCILEYATPLQTLFAMSQDAKAGFSREDRLEQAKLFCRTLEEILEDVPESRNNCRLIVYQEPTDGNSFSLSQEVLRHIRQEEKEEVT

SEQ ID NO: 26 - protein, 214 aa, Artificial Sequence
  Modified LPS Antibody Light Chain
NIVMTQSPDSLAVSLGERATISCKASENVGNSVSWYQQKPGQSPKPLIYGASNRYTGVPDRFSGSGSATDFTLTISSLQAEDVAVYHCGQSYSYPYTFGGGTKVEIKRTVAAPSVFIFPPSDEQLKSGTASVVCLLNNFYPREAKVQWKVDNALQSGNSQESVTEQDSKDSTYSLSSTLTLSKADYEKHKVYACEVTHQGLSSPVTKSFNRGEC

SEQ ID NO: 27 - protein, 451 aa, Artificial Sequence
  Modified LPS Antibody Heavy Chain
QVQLVQSGAEVKKPGASVKVSCKASGYTFTTYWINWVRQAPGQGLEWMGNIYPGTRSSNYNEKFKNRVTLTVDTSTSTAYMELSSLRSEDTAVYYCTRVYYDHVGYYFDYWGQGTLVTVSSASTKGPSVFPLAPSSKSTSGGTAALGCLVKDYFPEPVTVSWNSGALTSGVHTFPAVLQSSGLYSLSSVVTVPSSSLGTQTYICNVNHKPSNTKVDKRVEPKSCDKTHTCPPCPAPEAAGGPSVFLFPPKPKDTLMISRTPEVTCVVVDVSHEDPEVKFNWYVDGVEVHNAKTKPREEQYNSTYRVVSVLTVLHQDWLNGKEYKCKVSNKALPAPIEKTISKAKGQPREPQVYTLPPSREEMTKNQVSLTCLVKGFYPSDIAVEWESNGQPENNYKTTPPVLDSDGSFFLYSKLTVDKSRWQQGNVFSCSVMHEALHNHYTQKSLSLSPGK

SEQ ID NO: 28 - protein, 214 aa, Artificial Sequence
  Pertuzumab Light Chain
DIQMTQSPSSLSASVGDRVTITCKASQDVSIGVAWYQQKPGKAPKLLIYSASYRYTGVPSRFSGSGSGTDFTLTISSLQPEDFATYYCQQYYIYPYTFGQGTKVEIKRTVAAPSVFIFPPSDEQLKSGTASVVCLLNNFYPREAKVQWKVDNALQSGNSQESVTEQDSKDSTYSLSSTLTLSKADYEKHKVYACEVTHQGLSSPVTKSFNRGEC

SEQ ID NO: 29 - protein, 449 aa, Artificial Sequence
  Pertuzumab Heavy Chain
EVQLVESGGGLVQPGGSLRLSCAASGFTFTDYTMDWVRQAPGKGLEWVADVNPNSGGSIYNQRFKGRFTLSVDRSKNTLYLQMNSLRAEDTAVYYCARNLGPSFYFDYWGQGTLVTVSSASTKGPSVFPLAPSSKSTSGGTAALGCLVKDYFPEPVTVSWNSGALTSGVHTFPAVLQSSGLYSLSSVVTVPSSSLGTQTYICNVNHKPSNTKVDKKVEPKSCDKTHTCPPCPAPELLGGPSVFLFPPKPKDTLMISRTPEVTCVVVDVSHEDPEVKFNWYVDGVEVHNAKTKPREEQYNSTYRVVSVLTVLHQDWLNGKEYKCKVSNKALPAPIEKTISKAKGQPREPQVYTLPPSREEMTKNQVSLTCLVKGFYPSDIAVEWESNGQPENNYKTTPPVLDSDGSFFLYSKLTVDKSRWQQGNVFSCSVMHEALHNHYTQKSLSLSPGK

SEQ ID NO: 30 - protein, 449 aa, Artificial Sequence
  Modified HER2 Antibody2 Heavy Chain
EVQLVESGGGLVQPGGSLRLSCAASGFTFTDYTMDWVRQAPGKGLEWVADVNPNSGGSIYNQRFKGRFTLSVDRSKNTLYLQMNSLRAEDTAVYYCARNLGPSFYFDYWGQGTLVTVSSASTKGPSVFPLAPSSKSTSGGTAALGCLVKDYFPEPVTVSWNSGALTSGVHTFPAVLQSSGLYSLSSVVTVPSSSLGTQTYICNVNHKPSNTKVDKRVEPKSCDKTHTCPPCPAPEAAGGPSVFLFPPKPKDTLMISRTPEVTCVVVDVSHEDPEVKFNWYVDGVEVHNAKTKPREEQYNSTYRVVSVLTVLHQDWLNGKEYKCKVSNKALPAPIEKTISKAKGQPREPQVYTLPPSREEMTKNQVSLTCLVKGFYPSDIAVEWESNGQPENNYKTTPPVLDSDGSFFLYSKLTVDKSRWQQGNVFSCSVMHEALHNHYTQKSLSLSPGK

SEQ ID NO: 31 - protein, 218 aa, Artificial Sequence
  Anti-CD33 Antibody Light Chain
DIQLTQSPSTLSASVGDRVTITCRASESLDNYGIRFLTWFQQKPGKAPKLLMYAASNQGSGVPSRFSGSGSGTEFTLTISSLQPDDFATYYCQQTKEVPWSFGQGTKVEVKRTVAAPSVFIFPPSDEQLKSGTASVVCLLNNFYPREAKVQWKVDNALQSGNSQESVTEQDSKDSTYSLSSTLTLSKADYEKHKVYACEVTHQGLSSPVTKSFNRGEC

SEQ ID NO: 32 - protein, 446 aa, Artificial Sequence
  Anti-CD33 Antibody Heavy Chain
EVQLVQSGAEVKKPGSSVKVSCKASGYTITDSNIHWVRQAPGQSLEWIGYIYPYNGGTDYNQKFKNRATLTVDNPTNTAYMELSSLRSEDTAFYYCVNGNPWLAYWGQGTLVTVSSASTKGPSVFPLAPSSKSTSGGTAALGCLVKDYFPEPVTVSWNSGALTSGVHTFPAVLQSSGLYSLSSVVTVPSSSLGTQTYICNVNHKPSNTKVDKRVEPKSCDKTHTCPPCPAPEAAGGPSVFLFPPKPKDTLMISRTPEVTCVVVDVSHEDPEVKFNWYVDGVEVHNAKTKPREEQYNSTYRVVSVLTVLHQDWLNGKEYKCKVSNKALPAPIEKTISKAKGQPREPQVYTLPPSREEMTKNQVSLTCLVKGFYPSDIAVEWESNGQPENNYKTTPPVLDSDGSFFLYSKLTVDKSRWQQGNVFSCSVMHEALHNHYTQKSLSLSPGK

SEQ ID NO: 33 - protein, 219 aa, Artificial Sequence
  Anti-EphA2 Antibody Light Chain
DIVMTQSPLSLPVTPGEPASISCRSSQSIVHSSGITYLEWYLQKPGQSPQLLIYKVSNRFSGVPDRFSGSGSGTDFTLKISRVEAEDVGVYYCFQGSHVPYTFGQGTKVEIKRTVAAPSVFIFPPSDEQLKSGTASVVCLLNNFYPREAKVQWKVDNALQSGNSQESVTEQDSKDSTYSLSSTLTLSKADYEKHKVYACEVTHQGLSSPVTKSFNRGEC

SEQ ID NO: 34 - protein, 449 aa, Artificial Sequence
  Anti-EphA2 Antibody Heavy Chain
QVQLVQSGAEVKKPGASVKVSCKASGYTFIDYSMHWVRQAPGQGLEWMGWINTYTGEPTYSDDFKGRVTITADTSTSTAYLELSSLRSEDTAVYYCATYYRYERDFDYWGQGTLVTVSSASTKGPSVFPLAPSSKSTSGGTAALGCLVKDYFPEPVTVSWNSGALTSGVHTFPAVLQSSGLYSLSSVVTVPSSSLGTQTYICNVNHKPSNTKVDKRVEPKSCDKTHTCPPCPAPELLGGPSVFLFPPKPKDTLMISRTPEVTCVVVDVSHEDPEVKFNWYVDGVEVHNAKTKPREEQYNSTYRVVSVLTVLHQDWLNGKEYKCKVSNKALPAPIEKTISKAKGQPREPQVYTLPPSREEMTKNQVSLTCLVKGFYPSDIAVEWESNGQPENNYKTTPPVLDSDGSFFLYSKLTVDKSRWQQGNVFSCSVMHEALHNHYTQKSLSLSPGK

SEQ ID NO: 35 - protein, 213 aa, Artificial Sequence
  Anti-CDH6 Antibody Light Chain
DIQMTQSPSSLSASVGDRVTITCKASQNIYKNLAWYQQKPGKAPKLLIYDANTLQTGVPSRFSGSGSGSDFTLTISSLQPEDFATYFCQQYYSGWAFGQGTKVEIKRTVAAPSVFIFPPSDEQLKSGTASVVCLLNNFYPREAKVQWKVDNALQSGNSQESVTEQDSKDSTYSLSSTLTLSKADYEKHKVYACEVTHQGLSSPVTKSFNRGEC

SEQ ID NO: 36 - protein, 452 aa, Artificial Sequence
  Anti-CDH6 Antibody Heavy Chain
EVQLVQSGAEVKKPGASVKVSCKASGYTFTRNFMHWVRQAPGQGLEWMGWIYPGDGETEYAQKFQGRVTITADTSTSTAYMELSSLRSEDTAVYYCARGVYGGFAGGYFDFWGQGTLVTVSSASTKGPSVFPLAPSSKSTSGGTAALGCLVKDYFPEPVTVSWNSGALTSGVHTFPAVLQSSGLYSLSSVVTVPSSSLGTQTYICNVNHKPSNTKVDKRVEPKSCDKTHTCPPCPAPEAAGGPSVFLFPPKPKDTLMISRTPEVTCVVVDVSHEDPEVKFNWYVDGVEVHNAKTKPREEQYNSTYRVVSVLTVLHQDWLNGKEYKCKVSNKALGAPIEKTISKAKGQPREPQVYTLPPSREEMTKNQVSLTCLVKGFYPSDIAVEWESNGQPENNYKTTPPVLDSDGSFFLYSKLTVDKSRWQQGNVFSCSVMHEALHNHYTQKSLSLSPGK